European Patent Application EP 4 206 322 A2, published July 5, 2023. Title: POLYPEPTIDE AND METHOD FOR PRODUCING AMINO ACID DERIVATIVE USING SAME. Applicant: CHUGAI SEIYAKU KABUSHIKI KAISHA. Application EP. The sequence listing filed with the application follows.

SEQUENCE LISTING (62 sequences)

SEQ ID NO: 1 - protein, 332 aa, Pseudomonas putida KT2440
MRVPFTELQSLLQAIFQRHGCSEAVARVLAHNCASAQRDGAHSHGVFRMPGYVSTLASGWVDGQATPQVSDVAAGYVRVDAAGGFAQPALAAARELLVAKARSAGIAVLAIHNSHHFAALWPDVEPFAEEGLVALSVVNSMTCVVPHGARKPLFGTNPIAFAAPCAEHDPIVFDMATSAMAHGDVQIAARAGQQLPEGMGVDADGQPTTDPKAILEGGALLPFGGHKGSALSMMVELLAAALTGGHFSWEFDWSGHPGAKTPWTGQLIIVIDPGKAEGQRFAQRSRELVEHMQAVGLTRMPGERRYREREVAEEEGVAVTEQELKGLKELLG

SEQ ID NO: 2 - protein, 332 aa, synthetic construct
  REGION 1..332: note = H44X
  VARIANT 44: note = A, R, N, D, C, Q, E, G, I, L, K, M, F, P, S, T, W, Y or V
MRVPFTELQSLLQAIFQRHGCSEAVARVLAHNCASAQRDGAHSXGVFRMPGYVSTLASGWVDGQATPQVSDVAAGYVRVDAAGGFAQPALAAARELLVAKARSAGIAVLAIHNSHHFAALWPDVEPFAEEGLVALSVVNSMTCVVPHGARKPLFGTNPIAFAAPCAEHDPIVFDMATSAMAHGDVQIAARAGQQLPEGMGVDADGQPTTDPKAILEGGALLPFGGHKGSALSMMVELLAAALTGGHFSWEFDWSGHPGAKTPWTGQLIIVIDPGKAEGQRFAQRSRELVEHMQAVGLTRMPGERRYREREVAEEEGVAVTEQELKGLKELLG

SEQ ID NO: 3 - protein, 332 aa, synthetic construct
  REGION 1..332: note = R48X
  VARIANT 48: note = A, N, D, C, Q, E, G, H, I, L, K, M, F, P, S, T, W, Y or V
MRVPFTELQSLLQAIFQRHGCSEAVARVLAHNCASAQRDGAHSHGVFXMPGYVSTLASGWVDGQATPQVSDVAAGYVRVDAAGGFAQPALAAARELLVAKARSAGIAVLAIHNSHHFAALWPDVEPFAEEGLVALSVVNSMTCVVPHGARKPLFGTNPIAFAAPCAEHDPIVFDMATSAMAHGDVQIAARAGQQLPEGMGVDADGQPTTDPKAILEGGALLPFGGHKGSALSMMVELLAAALTGGHFSWEFDWSGHPGAKTPWTGQLIIVIDPGKAEGQRFAQRSRELVEHMQAVGLTRMPGERRYREREVAEEEGVAVTEQELKGLKELLG

SEQ ID NO: 4 - protein, 332 aa, synthetic construct
  REGION 1..332: note = F117X
  VARIANT 117: note = A, R, N, D, C, Q, E, G, H, I, L, K, M, P, S, T, W, Y or V
MRVPFTELQSLLQAIFQRHGCSEAVARVLAHNCASAQRDGAHSHGVFRMPGYVSTLASGWVDGQATPQVSDVAAGYVRVDAAGGFAQPALAAARELLVAKARSAGIAVLAIHNSHHXAALWPDVEPFAEEGLVALSVVNSMTCVVPHGARKPLFGTNPIAFAAPCAEHDPIVFDMATSAMAHGDVQIAARAGQQLPEGMGVDADGQPTTDPKAILEGGALLPFGGHKGSALSMMVELLAAALTGGHFSWEFDWSGHPGAKTPWTGQLIIVIDPGKAEGQRFAQRSRELVEHMQAVGLTRMPGERRYREREVAEEEGVAVTEQELKGLKELLG

SEQ ID NO: 5 - protein, 332 aa, synthetic construct
  REGION 1..332: note = S140X
  VARIANT 140: note = A, R, N, D, C, Q, E, G, H, I, L, K, M, F, P, T, W, Y or V
MRVPFTELQSLLQAIFQRHGCSEAVARVLAHNCASAQRDGAHSHGVFRMPGYVSTLASGWVDGQATPQVSDVAAGYVRVDAAGGFAQPALAAARELLVAKARSAGIAVLAIHNSHHFAALWPDVEPFAEEGLVALSVVNXMTCVVPHGARKPLFGTNPIAFAAPCAEHDPIVFDMATSAMAHGDVQIAARAGQQLPEGMGVDADGQPTTDPKAILEGGALLPFGGHKGSALSMMVELLAAALTGGHFSWEFDWSGHPGAKTPWTGQLIIVIDPGKAEGQRFAQRSRELVEHMQAVGLTRMPGERRYREREVAEEEGVAVTEQELKGLKELLG

SEQ ID NO: 6 - protein, 332 aa, synthetic construct
  REGION 1..332: note = M141X
  VARIANT 141: note = A, R, N, D, C, Q, E, G, H, I, L, K, F, P, S, T, W, Y or V
MRVPFTELQSLLQAIFQRHGCSEAVARVLAHNCASAQRDGAHSHGVFRMPGYVSTLASGWVDGQATPQVSDVAAGYVRVDAAGGFAQPALAAARELLVAKARSAGIAVLAIHNSHHFAALWPDVEPFAEEGLVALSVVNSXTCVVPHGARKPLFGTNPIAFAAPCAEHDPIVFDMATSAMAHGDVQIAARAGQQLPEGMGVDADGQPTTDPKAILEGGALLPFGGHKGSALSMMVELLAAALTGGHFSWEFDWSGHPGAKTPWTGQLIIVIDPGKAEGQRFAQRSRELVEHMQAVGLTRMPGERRYREREVAEEEGVAVTEQELKGLKELLG

SEQ ID NO: 7 - protein, 332 aa, synthetic construct
  REGION 1..332: note = T156X
  VARIANT 156: note = A, R, N, D, C, Q, E, G, H, I, L, K, M, F, P, S, W, Y or V
MRVPFTELQSLLQAIFQRHGCSEAVARVLAHNCASAQRDGAHSHGVFRMPGYVSTLASGWVDGQATPQVSDVAAGYVRVDAAGGFAQPALAAARELLVAKARSAGIAVLAIHNSHHFAALWPDVEPFAEEGLVALSVVNSMTCVVPHGARKPLFGXNPIAFAAPCAEHDPIVFDMATSAMAHGDVQIAARAGQQLPEGMGVDADGQPTTDPKAILEGGALLPFGGHKGSALSMMVELLAAALTGGHFSWEFDWSGHPGAKTPWTGQLIIVIDPGKAEGQRFAQRSRELVEHMQAVGLTRMPGERRYREREVAEEEGVAVTEQELKGLKELLG

SEQ ID NO: 8 - protein, 332 aa, synthetic construct
  REGION 1..332: note = H182X
  VARIANT 182: note = A, R, N, D, C, Q, E, G, I, L, K, M, F, P, S, T, W, Y or V
MRVPFTELQSLLQAIFQRHGCSEAVARVLAHNCASAQRDGAHSHGVFRMPGYVSTLASGWVDGQATPQVSDVAAGYVRVDAAGGFAQPALAAARELLVAKARSAGIAVLAIHNSHHFAALWPDVEPFAEEGLVALSVVNSMTCVVPHGARKPLFGTNPIAFAAPCAEHDPIVFDMATSAMAXGDVQIAARAGQQLPEGMGVDADGQPTTDPKAILEGGALLPFGGHKGSALSMMVELLAAALTGGHFSWEFDWSGHPGAKTPWTGQLIIVIDPGKAEGQRFAQRSRELVEHMQAVGLTRMPGERRYREREVAEEEGVAVTEQELKGLKELLG

SEQ ID NO: 9 - protein, 332 aa, synthetic construct
  REGION 1..332: note = G183X
  VARIANT 183: note = A, R, N, D, C, Q, E, H, I, L, K, M, F, P, S, T, W, Y or V
MRVPFTELQSLLQAIFQRHGCSEAVARVLAHNCASAQRDGAHSHGVFRMPGYVSTLASGWVDGQATPQVSDVAAGYVRVDAAGGFAQPALAAARELLVAKARSAGIAVLAIHNSHHFAALWPDVEPFAEEGLVALSVVNSMTCVVPHGARKPLFGTNPIAFAAPCAEHDPIVFDMATSAMAHXDVQIAARAGQQLPEGMGVDADGQPTTDPKAILEGGALLPFGGHKGSALSMMVELLAAALTGGHFSWEFDWSGHPGAKTPWTGQLIIVIDPGKAEGQRFAQRSRELVEHMQAVGLTRMPGERRYREREVAEEEGVAVTEQELKGLKELLG

SEQ ID NO: 10 - protein, 332 aa, synthetic construct
  REGION 1..332: note = Q186X
  VARIANT 186: note = A, R, N, D, C, E, G, H, I, L, K, M, F, P, S, T, W, Y or V
MRVPFTELQSLLQAIFQRHGCSEAVARVLAHNCASAQRDGAHSHGVFRMPGYVSTLASGWVDGQATPQVSDVAAGYVRVDAAGGFAQPALAAARELLVAKARSAGIAVLAIHNSHHFAALWPDVEPFAEEGLVALSVVNSMTCVVPHGARKPLFGTNPIAFAAPCAEHDPIVFDMATSAMAHGDVXIAARAGQQLPEGMGVDADGQPTTDPKAILEGGALLPFGGHKGSALSMMVELLAAALTGGHFSWEFDWSGHPGAKTPWTGQLIIVIDPGKAEGQRFAQRSRELVEHMQAVGLTRMPGERRYREREVAEEEGVAVTEQELKGLKELLG

SEQ ID NO: 11 - protein, 332 aa, synthetic construct
  REGION 1..332: note = W253X
  VARIANT 253: note = A, R, N, D, C, Q, E, G, H, I, L, K, M, F, P, S, T, Y or V
MRVPFTELQSLLQAIFQRHGCSEAVARVLAHNCASAQRDGAHSHGVFRMPGYVSTLASGWVDGQATPQVSDVAAGYVRVDAAGGFAQPALAAARELLVAKARSAGIAVLAIHNSHHFAALWPDVEPFAEEGLVALSVVNSMTCVVPHGARKPLFGTNPIAFAAPCAEHDPIVFDMATSAMAHGDVQIAARAGQQLPEGMGVDADGQPTTDPKAILEGGALLPFGGHKGSALSMMVELLAAALTGGHFSWEFDXSGHPGAKTPWTGQLIIVIDPGKAEGQRFAQRSRELVEHMQAVGLTRMPGERRYREREVAEEEGVAVTEQELKGLKELLG

SEQ ID NO: 12 - protein, 332 aa, synthetic construct
  REGION 1..332: note = K260X
  VARIANT 260: note = A, R, N, D, C, Q, E, G, H, I, L, M, F, P, S, T, W, Y or V
MRVPFTELQSLLQAIFQRHGCSEAVARVLAHNCASAQRDGAHSHGVFRMPGYVSTLASGWVDGQATPQVSDVAAGYVRVDAAGGFAQPALAAARELLVAKARSAGIAVLAIHNSHHFAALWPDVEPFAEEGLVALSVVNSMTCVVPHGARKPLFGTNPIAFAAPCAEHDPIVFDMATSAMAHGDVQIAARAGQQLPEGMGVDADGQPTTDPKAILEGGALLPFGGHKGSALSMMVELLAAALTGGHFSWEFDWSGHPGAXTPWTGQLIIVIDPGKAEGQRFAQRSRELVEHMQAVGLTRMPGERRYREREVAEEEGVAVTEQELKGLKELLG

SEQ ID NO: 13 - protein, 332 aa, synthetic construct
  REGION 1..332: note = P262X
  VARIANT 262: note = A, R, N, D, C, Q, E, G, H, I, L, K, M, F, S, T, W, Y or V
MRVPFTELQSLLQAIFQRHGCSEAVARVLAHNCASAQRDGAHSHGVFRMPGYVSTLASGWVDGQATPQVSDVAAGYVRVDAAGGFAQPALAAARELLVAKARSAGIAVLAIHNSHHFAALWPDVEPFAEEGLVALSVVNSMTCVVPHGARKPLFGTNPIAFAAPCAEHDPIVFDMATSAMAHGDVQIAARAGQQLPEGMGVDADGQPTTDPKAILEGGALLPFGGHKGSALSMMVELLAAALTGGHFSWEFDWSGHPGAKTXWTGQLIIVIDPGKAEGQRFAQRSRELVEHMQAVGLTRMPGERRYREREVAEEEGVAVTEQELKGLKELLG

SEQ ID NO: 14 - protein, 6 aa, synthetic construct
  REGION 1..6: note = His tag
HHHHHH

SEQ ID NO: 15 - protein, 34 aa, synthetic construct
  REGION 1..34: note = SBP tag
GTDEKTTGWRGGHVVEGLAGELEQLRARLEHHPQ

SEQ ID NO: 16 - protein, 43 aa, synthetic construct
  REGION 1..43: note = SBPtag-Linker-Histag
GTDEKTTGWRGGHVVEGLAGELEQLRARLEHHPQGGSHHHHHH

SEQ ID NO: 17 - protein, 375 aa, synthetic construct
  REGION 1..375: note = wild type NMAADH-SBPtag-Linker-Histag
MRVPFTELQSLLQAIFQRHGCSEAVARVLAHNCASAQRDGAHSHGVFRMPGYVSTLASGWVDGQATPQVSDVAAGYVRVDAAGGFAQPALAAARELLVAKARSAGIAVLAIHNSHHFAALWPDVEPFAEEGLVALSVVNSMTCVVPHGARKPLFGTNPIAFAAPCAEHDPIVFDMATSAMAHGDVQIAARAGQQLPEGMGVDADGQPTTDPKAILEGGALLPFGGHKGSALSMMVELLAAALTGGHFSWEFDWSGHPGAKTPWTGQLIIVIDPGKAEGQRFAQRSRELVEHMQAVGLTRMPGERRYREREVAEEEGVAVTEQELKGLKELLGGTDEKTTGWRGGHVVEGLAGELEQLRARLEHHPQGGSHHHHHH

SEQ ID NO: 18 - protein, 375 aa, synthetic construct
  REGION 1..375: note = M141V-SBPtag-Linker-Histag
MRVPFTELQSLLQAIFQRHGCSEAVARVLAHNCASAQRDGAHSHGVFRMPGYVSTLASGWVDGQATPQVSDVAAGYVRVDAAGGFAQPALAAARELLVAKARSAGIAVLAIHNSHHFAALWPDVEPFAEEGLVALSVVNSVTCVVPHGARKPLFGTNPIAFAAPCAEHDPIVFDMATSAMAHGDVQIAARAGQQLPEGMGVDADGQPTTDPKAILEGGALLPFGGHKGSALSMMVELLAAALTGGHFSWEFDWSGHPGAKTPWTGQLIIVIDPGKAEGQRFAQRSRELVEHMQAVGLTRMPGERRYREREVAEEEGVAVTEQELKGLKELLGGTDEKTTGWRGGHVVEGLAGELEQLRARLEHHPQGGSHHHHHH

SEQ ID NO: 19 - protein, 375 aa, synthetic construct
  REGION 1..375: note = M141Y-SBPtag-Linker-Histag
MRVPFTELQSLLQAIFQRHGCSEAVARVLAHNCASAQRDGAHSHGVFRMPGYVSTLASGWVDGQATPQVSDVAAGYVRVDAAGGFAQPALAAARELLVAKARSAGIAVLAIHNSHHFAALWPDVEPFAEEGLVALSVVNSYTCVVPHGARKPLFGTNPIAFAAPCAEHDPIVFDMATSAMAHGDVQIAARAGQQLPEGMGVDADGQPTTDPKAILEGGALLPFGGHKGSALSMMVELLAAALTGGHFSWEFDWSGHPGAKTPWTGQLIIVIDPGKAEGQRFAQRSRELVEHMQAVGLTRMPGERRYREREVAEEEGVAVTEQELKGLKELLGGTDEKTTGWRGGHVVEGLAGELEQLRARLEHHPQGGSHHHHHH

SEQ ID NO: 20 - protein, 375 aa, synthetic construct
  REGION 1..375: note = H182L-SBPtag-Linker-Histag
MRVPFTELQSLLQAIFQRHGCSEAVARVLAHNCASAQRDGAHSHGVFRMPGYVSTLASGWVDGQATPQVSDVAAGYVRVDAAGGFAQPALAAARELLVAKARSAGIAVLAIHNSHHFAALWPDVEPFAEEGLVALSVVNSMTCVVPHGARKPLFGTNPIAFAAPCAEHDPIVFDMATSAMALGDVQIAARAGQQLPEGMGVDADGQPTTDPKAILEGGALLPFGGHKGSALSMMVELLAAALTGGHFSWEFDWSGHPGAKTPWTGQLIIVIDPGKAEGQRFAQRSRELVEHMQAVGLTRMPGERRYREREVAEEEGVAVTEQELKGLKELLGGTDEKTTGWRGGHVVEGLAGELEQLRARLEHHPQGGSHHHHHH

SEQ ID NO: 21 - protein, 375 aa, synthetic construct
  REGION 1..375: note = W253H-SBPtag-Linker-Histag
MRVPFTELQSLLQAIFQRHGCSEAVARVLAHNCASAQRDGAHSHGVFRMPGYVSTLASGWVDGQATPQVSDVAAGYVRVDAAGGFAQPALAAARELLVAKARSAGIAVLAIHNSHHFAALWPDVEPFAEEGLVALSVVNSMTCVVPHGARKPLFGTNPIAFAAPCAEHDPIVFDMATSAMAHGDVQIAARAGQQLPEGMGVDADGQPTTDPKAILEGGALLPFGGHKGSALSMMVELLAAALTGGHFSWEFDHSGHPGAKTPWTGQLIIVIDPGKAEGQRFAQRSRELVEHMQAVGLTRMPGERRYREREVAEEEGVAVTEQELKGLKELLGGTDEKTTGWRGGHVVEGLAGELEQLRARLEHHPQGGSHHHHHH

SEQ ID NO: 22 - protein, 375 aa, synthetic construct
  REGION 1..375: note = K260E-SBPtag-Linker-Histag
MRVPFTELQSLLQAIFQRHGCSEAVARVLAHNCASAQRDGAHSHGVFRMPGYVSTLASGWVDGQATPQVSDVAAGYVRVDAAGGFAQPALAAARELLVAKARSAGIAVLAIHNSHHFAALWPDVEPFAEEGLVALSVVNSMTCVVPHGARKPLFGTNPIAFAAPCAEHDPIVFDMATSAMAHGDVQIAARAGQQLPEGMGVDADGQPTTDPKAILEGGALLPFGGHKGSALSMMVELLAAALTGGHFSWEFDWSGHPGAETPWTGQLIIVIDPGKAEGQRFAQRSRELVEHMQAVGLTRMPGERRYREREVAEEEGVAVTEQELKGLKELLGGTDEKTTGWRGGHVVEGLAGELEQLRARLEHHPQGGSHHHHHH

SEQ ID NO: 23 - protein, 332 aa, synthetic construct
  VARIANT 141: note = A, R, N, D, C, Q, E, G, H, I, L, K, F, P, S, T, W, Y or V
  VARIANT 182: note = A, R, N, D, C, Q, E, G, I, L, K, M, F, P, S, T, W, Y or V
MRVPFTELQSLLQAIFQRHGCSEAVARVLAHNCASAQRDGAHSHGVFRMPGYVSTLASGWVDGQATPQVSDVAAGYVRVDAAGGFAQPALAAARELLVAKARSAGIAVLAIHNSHHFAALWPDVEPFAEEGLVALSVVNSXTCVVPHGARKPLFGTNPIAFAAPCAEHDPIVFDMATSAMAXGDVQIAARAGQQLPEGMGVDADGQPTTDPKAILEGGALLPFGGHKGSALSMMVELLAAALTGGHFSWEFDWSGHPGAKTPWTGQLIIVIDPGKAEGQRFAQRSRELVEHMQAVGLTRMPGERRYREREVAEEEGVAVTEQELKGLKELLG

SEQ ID NO: 24 - protein, 332 aa, synthetic construct
  VARIANT 141: note = A, R, N, D, C, Q, E, G, H, I, L, K, F, P, S, T, W, Y or V
  VARIANT 253: note = A, R, N, D, C, Q, E, G, H, I, L, K, M, F, P, S, T, Y or V
MRVPFTELQSLLQAIFQRHGCSEAVARVLAHNCASAQRDGAHSHGVFRMPGYVSTLASGWVDGQATPQVSDVAAGYVRVDAAGGFAQPALAAARELLVAKARSAGIAVLAIHNSHHFAALWPDVEPFAEEGLVALSVVNSXTCVVPHGARKPLFGTNPIAFAAPCAEHDPIVFDMATSAMAHGDVQIAARAGQQLPEGMGVDADGQPTTDPKAILEGGALLPFGGHKGSALSMMVELLAAALTGGHFSWEFDXSGHPGAKTPWTGQLIIVIDPGKAEGQRFAQRSRELVEHMQAVGLTRMPGERRYREREVAEEEGVAVTEQELKGLKELLG

SEQ ID NO: 25 - protein, 332 aa, synthetic construct
  VARIANT 141: note = A, R, N, D, C, Q, E, G, H, I, L, K, F, P, S, T, W, Y or V
  VARIANT 260: note = A, R, N, D, C, Q, E, G, H, I, L, M, F, P, S, T, W, Y or V
MRVPFTELQSLLQAIFQRHGCSEAVARVLAHNCASAQRDGAHSHGVFRMPGYVSTLASGWVDGQATPQVSDVAAGYVRVDAAGGFAQPALAAARELLVAKARSAGIAVLAIHNSHHFAALWPDVEPFAEEGLVALSVVNSXTCVVPHGARKPLFGTNPIAFAAPCAEHDPIVFDMATSAMAHGDVQIAARAGQQLPEGMGVDADGQPTTDPKAILEGGALLPFGGHKGSALSMMVELLAAALTGGHFSWEFDWSGHPGAXTPWTGQLIIVIDPGKAEGQRFAQRSRELVEHMQAVGLTRMPGERRYREREVAEEEGVAVTEQELKGLKELLG

SEQ ID NO: 26 - protein, 332 aa, synthetic construct
  VARIANT 182: note = A, R, N, D, C, Q, E, G, I, L, K, M, F, P, S, T, W, Y or V
  VARIANT 253: note = A, R, N, D, C, Q, E, G, H, I, L, K, M, F, P, S, T, Y or V
MRVPFTELQSLLQAIFQRHGCSEAVARVLAHNCASAQRDGAHSHGVFRMPGYVSTLASGWVDGQATPQVSDVAAGYVRVDAAGGFAQPALAAARELLVAKARSAGIAVLAIHNSHHFAALWPDVEPFAEEGLVALSVVNSMTCVVPHGARKPLFGTNPIAFAAPCAEHDPIVFDMATSAMAXGDVQIAARAGQQLPEGMGVDADGQPTTDPKAILEGGALLPFGGHKGSALSMMVELLAAALTGGHFSWEFDXSGHPGAKTPWTGQLIIVIDPGKAEGQRFAQRSRELVEHMQAVGLTRMPGERRYREREVAEEEGVAVTEQELKGLKELLG

SEQ ID NO: 27 - protein, 332 aa, synthetic construct
  VARIANT 182: note = A, R, N, D, C, Q, E, G, I, L, K, M, F, P, S, T, W, Y or V
  VARIANT 260: note = A, R, N, D, C, Q, E, G, H, I, L, M, F, P, S, T, W, Y or V
MRVPFTELQSLLQAIFQRHGCSEAVARVLAHNCASAQRDGAHSHGVFRMPGYVSTLASGWVDGQATPQVSDVAAGYVRVDAAGGFAQPALAAARELLVAKARSAGIAVLAIHNSHHFAALWPDVEPFAEEGLVALSVVNSMTCVVPHGARKPLFGTNPIAFAAPCAEHDPIVFDMATSAMAXGDVQIAARAGQQLPEGMGVDADGQPTTDPKAILEGGALLPFGGHKGSALSMMVELLAAALTGGHFSWEFDWSGHPGAXTPWTGQLIIVIDPGKAEGQRFAQRSRELVEHMQAVGLTRMPGERRYREREVAEEEGVAVTEQELKGLKELLG

SEQ ID NO: 28 - protein, 332 aa, synthetic construct
  VARIANT 253: note = A, R, N, D, C, Q, E, G, H, I, L, K, M, F, P, S, T, Y or V
  VARIANT 260: note = A, R, N, D, C, Q, E, G, H, I, L, M, F, P, S, T, W, Y or V
MRVPFTELQSLLQAIFQRHGCSEAVARVLAHNCASAQRDGAHSHGVFRMPGYVSTLASGWVDGQATPQVSDVAAGYVRVDAAGGFAQPALAAARELLVAKARSAGIAVLAIHNSHHFAALWPDVEPFAEEGLVALSVVNSMTCVVPHGARKPLFGTNPIAFAAPCAEHDPIVFDMATSAMAHGDVQIAARAGQQLPEGMGVDADGQPTTDPKAILEGGALLPFGGHKGSALSMMVELLAAALTGGHFSWEFDXSGHPGAXTPWTGQLIIVIDPGKAEGQRFAQRSRELVEHMQAVGLTRMPGERRYREREVAEEEGVAVTEQELKGLKELLG

SEQ ID NO: 29 - protein, 332 aa, synthetic construct
  VARIANT 117: note = A, R, N, D, C, Q, E, G, H, I, L, K, M, P, S, T, W, Y or V
  VARIANT 141: note = A, R, N, D, C, Q, E, G, H, I, L, K, F, P, S, T, W, Y or V
MRVPFTELQSLLQAIFQRHGCSEAVARVLAHNCASAQRDGAHSHGVFRMPGYVSTLASGWVDGQATPQVSDVAAGYVRVDAAGGFAQPALAAARELLVAKARSAGIAVLAIHNSHHXAALWPDVEPFAEEGLVALSVVNSXTCVVPHGARKPLFGTNPIAFAAPCAEHDPIVFDMATSAMAHGDVQIAARAGQQLPEGMGVDADGQPTTDPKAILEGGALLPFGGHKGSALSMMVELLAAALTGGHFSWEFDWSGHPGAKTPWTGQLIIVIDPGKAEGQRFAQRSRELVEHMQAVGLTRMPGERRYREREVAEEEGVAVTEQELKGLKELLG

SEQ ID NO: 30 - protein, 332 aa, synthetic construct
  VARIANT 156: note = A, R, N, D, C, Q, E, G, H, I, L, K, M, F, P, S, W, Y or V
  VARIANT 186: note = A, R, N, D, C, E, G, H, I, L, K, M, F, P, S, T, W, Y or V
MRVPFTELQSLLQAIFQRHGCSEAVARVLAHNCASAQRDGAHSHGVFRMPGYVSTLASGWVDGQATPQVSDVAAGYVRVDAAGGFAQPALAAARELLVAKARSAGIAVLAIHNSHHFAALWPDVEPFAEEGLVALSVVNSMTCVVPHGARKPLFGXNPIAFAAPCAEHDPIVFDMATSAMAHGDVXIAARAGQQLPEGMGVDADGQPTTDPKAILEGGALLPFGGHKGSALSMMVELLAAALTGGHFSWEFDWSGHPGAKTPWTGQLIIVIDPGKAEGQRFAQRSRELVEHMQAVGLTRMPGERRYREREVAEEEGVAVTEQELKGLKELLG

SEQ ID NO: 31 - protein, 332 aa, synthetic construct
  VARIANT 141: note = A, R, N, D, C, Q, E, G, H, I, L, K, F, P, S, T, W, Y or V
  VARIANT 253: note = A, R, N, D, C, Q, E, G, H, I, L, K, M, F, P, S, T, Y or V
  VARIANT 260: note = A, R, N, D, C, Q, E, G, H, I, L, M, F, P, S, T, W, Y or V
MRVPFTELQSLLQAIFQRHGCSEAVARVLAHNCASAQRDGAHSHGVFRMPGYVSTLASGWVDGQATPQVSDVAAGYVRVDAAGGFAQPALAAARELLVAKARSAGIAVLAIHNSHHFAALWPDVEPFAEEGLVALSVVNSXTCVVPHGARKPLFGTNPIAFAAPCAEHDPIVFDMATSAMAHGDVQIAARAGQQLPEGMGVDADGQPTTDPKAILEGGALLPFGGHKGSALSMMVELLAAALTGGHFSWEFDXSGHPGAXTPWTGQLIIVIDPGKAEGQRFAQRSRELVEHMQAVGLTRMPGERRYREREVAEEEGVAVTEQELKGLKELLG

SEQ ID NO: 32 - protein, 332 aa, synthetic construct
  VARIANT 182: note = A, R, N, D, C, Q, E, G, I, L, K, M, F, P, S, T, W, Y or V
  VARIANT 253: note = A, R, N, D, C, Q, E, G, H, I, L, K, M, F, P, S, T, Y or V
  VARIANT 260: note = A, R, N, D, C, Q, E, G, H, I, L, M, F, P, S, T, W, Y or V
MRVPFTELQSLLQAIFQRHGCSEAVARVLAHNCASAQRDGAHSHGVFRMPGYVSTLASGWVDGQATPQVSDVAAGYVRVDAAGGFAQPALAAARELLVAKARSAGIAVLAIHNSHHFAALWPDVEPFAEEGLVALSVVNSMTCVVPHGARKPLFGTNPIAFAAPCAEHDPIVFDMATSAMAXGDVQIAARAGQQLPEGMGVDADGQPTTDPKAILEGGALLPFGGHKGSALSMMVELLAAALTGGHFSWEFDXSGHPGAXTPWTGQLIIVIDPGKAEGQRFAQRSRELVEHMQAVGLTRMPGERRYREREVAEEEGVAVTEQELKGLKELLG

SEQ ID NO: 33 - protein, 332 aa, synthetic construct
  VARIANT 141: note = A, R, N, D, C, Q, E, G, H, I, L, K, F, P, S, T, W, Y or V
  VARIANT 182: note = A, R, N, D, C, Q, E, G, I, L, K, M, F, P, S, T, W, Y or V
  VARIANT 260: note = A, R, N, D, C, Q, E, G, H, I, L, M, F, P, S, T, W, Y or V
MRVPFTELQSLLQAIFQRHGCSEAVARVLAHNCASAQRDGAHSHGVFRMPGYVSTLASGWVDGQATPQVSDVAAGYVRVDAAGGFAQPALAAARELLVAKARSAGIAVLAIHNSHHFAALWPDVEPFAEEGLVALSVVNSXTCVVPHGARKPLFGTNPIAFAAPCAEHDPIVFDMATSAMAXGDVQIAARAGQQLPEGMGVDADGQPTTDPKAILEGGALLPFGGHKGSALSMMVELLAAALTGGHFSWEFDWSGHPGAXTPWTGQLIIVIDPGKAEGQRFAQRSRELVEHMQAVGLTRMPGERRYREREVAEEEGVAVTEQELKGLKELLG

SEQ ID NO: 34 - protein, 332 aa, synthetic construct
  VARIANT 141: note = A, R, N, D, C, Q, E, G, H, I, L, K, F, P, S, T, W, Y or V
  VARIANT 182: note = A, R, N, D, C, Q, E, G, I, L, K, M, F, P, S, T, W, Y or V
  VARIANT 253: note = A, R, N, D, C, Q, E, G, H, I, L, K, M, F, P, S, T, Y or V
MRVPFTELQSLLQAIFQRHGCSEAVARVLAHNCASAQRDGAHSHGVFRMPGYVSTLASGWVDGQATPQVSDVAAGYVRVDAAGGFAQPALAAARELLVAKARSAGIAVLAIHNSHHFAALWPDVEPFAEEGLVALSVVNSXTCVVPHGARKPLFGTNPIAFAAPCAEHDPIVFDMATSAMAXGDVQIAARAGQQLPEGMGVDADGQPTTDPKAILEGGALLPFGGHKGSALSMMVELLAAALTGGHFSWEFDXSGHPGAKTPWTGQLIIVIDPGKAEGQRFAQRSRELVEHMQAVGLTRMPGERRYREREVAEEEGVAVTEQELKGLKELLG

SEQ ID NO: 35 - protein, 332 aa, synthetic construct
  VARIANT 117: note = A, R, N, D, C, Q, E, G, H, I, L, K, M, P, S, T, W, Y or V
  VARIANT 141: note = A, R, N, D, C, Q, E, G, H, I, L, K, F, P, S, T, W, Y or V
  VARIANT 260: note = A, R, N, D, C, Q, E, G, H, I, L, M, F, P, S, T, W, Y or V
MRVPFTELQSLLQAIFQRHGCSEAVARVLAHNCASAQRDGAHSHGVFRMPGYVSTLASGWVDGQATPQVSDVAAGYVRVDAAGGFAQPALAAARELLVAKARSAGIAVLAIHNSHHXAALWPDVEPFAEEGLVALSVVNSXTCVVPHGARKPLFGTNPIAFAAPCAEHDPIVFDMATSAMAHGDVQIAARAGQQLPEGMGVDADGQPTTDPKAILEGGALLPFGGHKGSALSMMVELLAAALTGGHFSWEFDWSGHPGAXTPWTGQLIIVIDPGKAEGQRFAQRSRELVEHMQAVGLTRMPGERRYREREVAEEEGVAVTEQELKGLKELLG

SEQ ID NO: 36 - protein, 375 aa, synthetic construct
MRVPFTELQSLLQAIFQRHGCSEAVARVLAHNCASAQRDGAHSHGVFRMPGYVSTLASGWVDGQATPQVSDVAAGYVRVDAAGGFAQPALAAARELLVAKARSAGIAVLAIHNSHHFAALWPDVEPFAEEGLVALSVVNSATCVVPHGARKPLFGTNPIAFAAPCAEHDPIVFDMATSAMAHGDVQIAARAGQQLPEGMGVDADGQPTTDPKAILEGGALLPFGGHKGSALSMMVELLAAALTGGHFSWEFDWSGHPGAETPWTGQLIIVIDPGKAEGQRFAQRSRELVEHMQAVGLTRMPGERRYREREVAEEEGVAVTEQELKGLKELLGGTDEKTTGWRGGHVVEGLAGELEQLRARLEHHPQGGSHHHHHH

SEQ ID NO: 37 - protein, 375 aa, synthetic construct
MRVPFTELQSLLQAIFQRHGCSEAVARVLAHNCASAQRDGAHSHGVFRMPGYVSTLASGWVDGQATPQVSDVAAGYVRVDAAGGFAQPALAAARELLVAKARSAGIAVLAIHNSHHFAALWPDVEPFAEEGLVALSVVNSATCVVPHGARKPLFGTNPIAFAAPCAEHDPIVFDMATSAMAHGDVQIAARAGQQLPEGMGVDADGQPTTDPKAILEGGALLPFGGHKGSALSMMVELLAAALTGGHFSWEFDWSGHPGAQTPWTGQLIIVIDPGKAEGQRFAQRSRELVEHMQAVGLTRMPGERRYREREVAEEEGVAVTEQELKGLKELLGGTDEKTTGWRGGHVVEGLAGELEQLRARLEHHPQGGSHHHHHH

SEQ ID NO: 38 - protein, 375 aa, synthetic construct
MRVPFTELQSLLQAIFQRHGCSEAVARVLAHNCASAQRDGAHSHGVFRMPGYVSTLASGWVDGQATPQVSDVAAGYVRVDAAGGFAQPALAAARELLVAKARSAGIAVLAIHNSHHFAALWPDVEPFAEEGLVALSVVNSYTCVVPHGARKPLFGTNPIAFAAPCAEHDPIVFDMATSAMAHGDVQIAARAGQQLPEGMGVDADGQPTTDPKAILEGGALLPFGGHKGSALSMMVELLAAALTGGHFSWEFDWSGHPGAETPWTGQLIIVIDPGKAEGQRFAQRSRELVEHMQAVGLTRMPGERRYREREVAEEEGVAVTEQELKGLKELLGGTDEKTTGWRGGHVVEGLAGELEQLRARLEHHPQGGSHHHHHH

SEQ ID NO: 39 - protein, 375 aa, synthetic construct
MRVPFTELQSLLQAIFQRHGCSEAVARVLAHNCASAQRDGAHSHGVFRMPGYVSTLASGWVDGQATPQVSDVAAGYVRVDAAGGFAQPALAAARELLVAKARSAGIAVLAIHNSHHFAALWPDVEPFAEEGLVALSVVNSVTCVVPHGARKPLFGTNPIAFAAPCAEHDPIVFDMATSAMAHGDVQIAARAGQQLPEGMGVDADGQPTTDPKAILEGGALLPFGGHKGSALSMMVELLAAALTGGHFSWEFDWSGHPGAETPWTGQLIIVIDPGKAEGQRFAQRSRELVEHMQAVGLTRMPGERRYREREVAEEEGVAVTEQELKGLKELLGGTDEKTTGWRGGHVVEGLAGELEQLRARLEHHPQGGSHHHHHH

SEQ ID NO: 40 - protein, 375 aa, synthetic construct; identical to SEQ ID NO: 39

SEQ ID NO: 41 - protein, 375 aa, synthetic construct
MRVPFTELQSLLQAIFQRHGCSEAVARVLAHNCASAQRDGAHSHGVFRMPGYVSTLASGWVDGQATPQVSDVAAGYVRVDAAGGFAQPALAAARELLVAKARSAGIAVLAIHNSHHFAALWPDVEPFAEEGLVALSVVNSMTCVVPHGARKPLFGTNPIAFAAPCAEHDPIVFDMATSAMALGDVQIAARAGQQLPEGMGVDADGQPTTDPKAILEGGALLPFGGHKGSALSMMVELLAAALTGGHFSWEFDWSGHPGAQTPWTGQLIIVIDPGKAEGQRFAQRSRELVEHMQAVGLTRMPGERRYREREVAEEEGVAVTEQELKGLKELLGGTDEKTTGWRGGHVVEGLAGELEQLRARLEHHPQGGSHHHHHH

SEQ ID NO: 42 - protein, 375 aa, synthetic construct
MRVPFTELQSLLQAIFQRHGCSEAVARVLAHNCASAQRDGAHSHGVFRMPGYVSTLASGWVDGQATPQVSDVAAGYVRVDAAGGFAQPALAAARELLVAKARSAGIAVLAIHNSHHFAALWPDVEPFAEEGLVALSVVNSMTCVVPHGARKPLFGTNPIAFAAPCAEHDPIVFDMATSAMAMGDVQIAARAGQQLPEGMGVDADGQPTTDPKAILEGGALLPFGGHKGSALSMMVELLAAALTGGHFSWEFDWSGHPGAETPWTGQLIIVIDPGKAEGQRFAQRSRELVEHMQAVGLTRMPGERRYREREVAEEEGVAVTEQELKGLKELLGGTDEKTTGWRGGHVVEGLAGELEQLRARLEHHPQGGSHHHHHH

SEQ ID NO: 43 - protein, 375 aa, synthetic construct
MRVPFTELQSLLQAIFQRHGCSEAVARVLAHNCASAQRDGAHSHGVFRMPGYVSTLASGWVDGQATPQVSDVAAGYVRVDAAGGFAQPALAAARELLVAKARSAGIAVLAIHNSHHFAALWPDVEPFAEEGLVALSVVNSMTCVVPHGARKPLFGTNPIAFAAPCAEHDPIVFDMATSAMAMGDVQIAARAGQQLPEGMGVDADGQPTTDPKAILEGGALLPFGGHKGSALSMMVELLAAALTGGHFSWEFDWSGHPGAQTPWTGQLIIVIDPGKAEGQRFAQRSRELVEHMQAVGLTRMPGERRYREREVAEEEGVAVTEQELKGLKELLGGTDEKTTGWRGGHVVEGLAGELEQLRARLEHHPQGGSHHHHHH

SEQ ID NO: 44 - protein, 375 aa, synthetic construct
MRVPFTELQSLLQAIFQRHGCSEAVARVLAHNCASAQRDGAHSHGVFRMPGYVSTLASGWVDGQATPQVSDVAAGYVRVDAAGGFAQPALAAARELLVAKARSAGIAVLAIHNSHHFAALWPDVEPFAEEGLVALSVVNSMTCVVPHGARKPLFGTNPIAFAAPCAEHDPIVFDMATSAMAHGDVQIAARAGQQLPEGMGVDADGQPTTDPKAILEGGALLPFGGHKGSALSMMVELLAAALTGGHFSWEFDHSGHPGAETPWTGQLIIVIDPGKAEGQRFAQRSRELVEHMQAVGLTRMPGERRYREREVAEEEGVAVTEQELKGLKELLGGTDEKTTGWRGGHVVEGLAGELEQLRARLEHHPQGGSHHHHHH

SEQ ID NO: 45 - protein, 375 aa, synthetic construct
MRVPFTELQSLLQAIFQRHGCSEAVARVLAHNCASAQRDGAHSHGVFRMPGYVSTLASGWVDGQATPQVSDVAAGYVRVDAAGGFAQPALAAARELLVAKARSAGIAVLAIHNSHHFAALWPDVEPFAEEGLVALSVVNSITCVVPHGARKPLFGTNPIAFAAPCAEHDPIVFDMATSAMAHGDVQIAARAGQQLPEGMGVDADGQPTTDPKAILEGGALLPFGGHKGSALSMMVELLAAALTGGHFSWEFDHSGHPGAETPWTGQLIIVIDPGKAEGQRFAQRSRELVEHMQAVGLTRMPGERRYREREVAEEEGVAVTEQELKGLKELLGGTDEKTTGWRGGHVVEGLAGELEQLRARLEHHPQGGSHHHHHH

SEQ ID NO: 46 - protein, 375 aa, synthetic construct
MRVPFTELQSLLQAIFQRHGCSEAVARVLAHNCASAQRDGAHSHGVFRMPGYVSTLASGWVDGQATPQVSDVAAGYVRVDAAGGFAQPALAAARELLVAKARSAGIAVLAIHNSHHFAALWPDVEPFAEEGLVALSVVNSITCVVPHGARKPLFGTNPIAFAAPCAEHDPIVFDMATSAMAHGDVQIAARAGQQLPEGMGVDADGQPTTDPKAILEGGALLPFGGHKGSALSMMVELLAAALTGGHFSWEFDHSGHPGAQTPWTGQLIIVIDPGKAEGQRFAQRSRELVEHMQAVGLTRMPGERRYREREVAEEEGVAVTEQELKGLKELLGGTDEKTTGWRGGHVVEGLAGELEQLRARLEHHPQGGSHHHHHH

SEQ ID NO: 47 - protein, 375 aa, synthetic construct
MRVPFTELQSLLQAIFQRHGCSEAVARVLAHNCASAQRDGAHSHGVFRMPGYVSTLASGWVDGQATPQVSDVAAGYVRVDAAGGFAQPALAAARELLVAKARSAGIAVLAIHNSHHFAALWPDVEPFAEEGLVALSVVNSVTCVVPHGARKPLFGTNPIAFAAPCAEHDPIVFDMATSAMALGDVQIAARAGQQLPEGMGVDADGQPTTDPKAILEGGALLPFGGHKGSALSMMVELLAAALTGGHFSWEFDWSGHPGAETPWTGQLIIVIDPGKAEGQRFAQRSRELVEHMQAVGLTRMPGERRYREREVAEEEGVAVTEQELKGLKELLGGTDEKTTGWRGGHVVEGLAGELEQLRARLEHHPQGGSHHHHHH

SEQ ID NO: 48 - protein, 375 aa, synthetic construct
MRVPFTELQSLLQAIFQRHGCSEAVARVLAHNCASAQRDGAHSHGVFRMPGYVSTLASGWVDGQATPQVSDVAAGYVRVDAAGGFAQPALAAARELLVAKARSAGIAVLAIHNSHHFAALWPDVEPFAEEGLVALSVVNSVTCVVPHGARKPLFGTNPIAFAAPCAEHDPIVFDMATSAMALGDVQIAARAGQQLPEGMGVDADGQPTTDPKAILEGGALLPFGGHKGSALSMMVELLAAALTGGHFSWEFDWSGHPGAQTPWTGQLIIVIDPGKAEGQRFAQRSRELVEHMQAVGLTRMPGERRYREREVAEEEGVAVTEQELKGLKELLGGTDEKTTGWRGGHVVEGLAGELEQLRARLEHHPQGGSHHHHHH

SEQ ID NO: 49 - protein, 375 aa, synthetic construct
MRVPFTELQSLLQAIFQRHGCSEAVARVLAHNCASAQRDGAHSHGVFRMPGYVSTLASGWVDGQATPQVSDVAAGYVRVDAAGGFAQPALAAARELLVAKARSAGIAVLAIHNSHHFAALWPDVEPFAEEGLVALSVVNSVTCVVPHGARKPLFGTNPIAFAAPCAEHDPIVFDMATSAMAMGDVQIAARAGQQLPEGMGVDADGQPTTDPKAILEGGALLPFGGHKGSALSMMVELLAAALTGGHFSWEFDWSGHPGAETPWTGQLIIVIDPGKAEGQRFAQRSRELVEHMQAVGLTRMPGERRYREREVAEEEGVAVTEQELKGLKELLGGTDEKTTGWRGGHVVEGLAGELEQLRARLEHHPQGGSHHHHHH

SEQ ID NO: 50 - protein, 375 aa, synthetic construct
MRVPFTELQSLLQAIFQRHGCSEAVARVLAHNCASAQRDGAHSHGVFRMPGYVSTLASGWVDGQATPQVSDVAAGYVRVDAAGGFAQPALAAARELLVAKARSAGIAVLAIHNSHHFAALWPDVEPFAEEGLVALSVVNSVTCVVPHGARKPLFGTNPIAFAAPCAEHDPIVFDMATSAMAHGDVQIAARAGQQLPEGMGVDADGQPTTDPKAILEGGALLPFGGHKGSALSMMVELLAAALTGGHFSWEFDHSGHPGAQTPWTGQLIIVIDPGKAEGQRFAQRSRELVEHMQAVGLTRMPGERRYREREVAEEEGVAVTEQELKGLKELLGGTDEKTTGWRGGHVVEGLAGELEQLRARLEHHPQGGSHHHHHH

SEQ ID NO: 51 - protein, 375 aa, synthetic construct
MRVPFTELQSLLQAIFQRHGCSEAVARVLAHNCASAQRDGAHSHGVFRMPGYVSTLASGWVDGQATPQVSDVAAGYVRVDAAGGFAQPALAAARELLVAKARSAGIAVLAIHNSHHFAALWPDVEPFAEEGLVALSVVNSVTCVVPHGARKPLFGTNPIAFAAPCAEHDPIVFDMATSAMAHGDVQIAARAGQQLPEGMGVDADGQPTTDPKAILEGGALLPFGGHKGSALSMMVELLAAALTGGHFSWEFDLSGHPGAQTPWTGQLIIVIDPGKAEGQRFAQRSRELVEHMQAVGLTRMPGERRYREREVAEEEGVAVTEQELKGLKELLGGTDEKTTGWRGGHVVEGLAGELEQLRARLEHHPQGGSHHHHHH

SEQ ID NO: 52 - protein, 375 aa, synthetic construct
MRVPFTELQSLLQAIFQRHGCSEAVARVLAHNCASAQRDGAHSHGVFRMPGYVSTLASGWVDGQATPQVSDVAAGYVRVDAAGGFAQPALAAARELLVAKARSAGIAVLAIHNSHHFAALWPDVEPFAEEGLVALSVVNSVTCVVPHGARKPLFGTNPIAFAAPCAEHDPIVFDMATSAMAHGDVQIAARAGQQLPEGMGVDADGQPTTDPKAILEGGALLPFGGHKGSALSMMVELLAAALTGGHFSWEFDMSGHPGAETPWTGQLIIVIDPGKAEGQRFAQRSRELVEHMQAVGLTRMPGERRYREREVAEEEGVAVTEQELKGLKELLGGTDEKTTGWRGGHVVEGLAGELEQLRARLEHHPQGGSHHHHHH

SEQ ID NO: 53 - protein, 375 aa, synthetic construct
MRVPFTELQSLLQAIFQRHGCSEAVARVLAHNCASAQRDGAHSHGVFRMPGYVSTLASGWVDGQATPQVSDVAAGYVRVDAAGGFAQPALAAARELLVAKARSAGIAVLAIHNSHHFAALWPDVEPFAEEGLVALSVVNSVTCVVPHGARKPLFGTNPIAFAAPCAEHDPIVFDMATSAMAHGDVQIAARAGQQLPEGMGVDADGQPTTDPKAILEGGALLPFGGHKGSALSMMVELLAAALTGGHFSWEFDQSGHPGAETPWTGQLIIVIDPGKAEGQRFAQRSRELVEHMQAVGLTRMPGERRYREREVAEEEGVAVTEQELKGLKELLGGTDEKTTGWRGGHVVEGLAGELEQLRARLEHHPQGGSHHHHHH

SEQ ID NO: 54 - protein, 375 aa, synthetic construct
MRVPFTELQSLLQAIFQRHGCSEAVARVLAHNCASAQRDGAHSHGVFRMPGYVSTLASGWVDGQATPQVSDVAAGYVRVDAAGGFAQPALAAARELLVAKARSAGIAVLAIHNSHHFAALWPDVEPFAEEGLVALSVVNSVTCVVPHGARKPLFGTNPIAFAAPCAEHDPIVFDMATSAMAHGDVQIAARAGQQLPEGMGVDADGQPTTDPKAILEGGALLPFGGHKGSALSMMVELLAAALTGGHFSWEFDMSGHPGAQTPWTGQLIIVIDPGKAEGQRFAQRSRELVEHMQAVGLTRMPGERRYREREVAEEEGVAVTEQELKGLKELLGGTDEKTTGWRGGHVVEGLAGELEQLRARLEHHPQGGSHHHHHH

SEQ ID NO: 55 - protein, 375 aa, synthetic construct
MRVPFTELQSLLQAIFQRHGCSEAVARVLAHNCASAQRDGAHSHGVFRMPGYVSTLASGWVDGQATPQVSDVAAGYVRVDAAGGFAQPALAAARELLVAKARSAGIAVLAIHNSHHFAALWPDVEPFAEEGLVALSVVNSVTCVVPHGARKPLFGTNPIAFAAPCAEHDPIVFDMATSAMAHGDVQIAARAGQQLPEGMGVDADGQPTTDPKAILEGGALLPFGGHKGSALSMMVELLAAALTGGHFSWEFDQSGHPGAQTPWTGQLIIVIDPGKAEGQRFAQRSRELVEHMQAVGLTRMPGERRYREREVAEEEGVAVTEQELKGLKELLGGTDEKTTGWRGGHVVEGLAGELEQLRARLEHHPQGGSHHHHHH

SEQ ID NO: 56 - protein, 375 aa, synthetic construct
MRVPFTELQSLLQAIFQRHGCSEAVARVLAHNCASAQRDGAHSHGVFRMPGYVSTLASGWVDGQATPQVSDVAAGYVRVDAAGGFAQPALAAARELLVAKARSAGIAVLAIHNSHHFAALWPDVEPFAEEGLVALSVVNSYTCVVPHGARKPLFGTNPIAFAAPCAEHDPIVFDMATSAMALGDVQIAARAGQQLPEGMGVDADGQPTTDPKAILEGGALLPFGGHKGSALSMMVELLAAALTGGHFSWEFDWSGHPGAETPWTGQLIIVIDPGKAEGQRFAQRSRELVEHMQAVGLTRMPGERRYREREVAEEEGVAVTEQELKGLKELLGGTDEKTTGWRGGHVVEGLAGELEQLRARLEHHPQGGSHHHHHH

SEQ ID NO: 57 - protein, 375 aa, synthetic construct
MRVPFTELQSLLQAIFQRHGCSEAVARVLAHNCASAQRDGAHSHGVFRMPGYVSTLASGWVDGQATPQVSDVAAGYVRVDAAGGFAQPALAAARELLVAKARSAGIAVLAIHNSHHFAALWPDVEPFAEEGLVALSVVNSYTCVVPHGARKPLFGTNPIAFAAPCAEHDPIVFDMATSAMALGDVQIAARAGQQLPEGMGVDADGQPTTDPKAILEGGALLPFGGHKGSALSMMVELLAAALTGGHFSWEFDWSGHPGAQTPWTGQLIIVIDPGKAEGQRFAQRSRELVEHMQAVGLTRMPGERRYREREVAEEEGVAVTEQELKGLKELLGGTDEKTTGWRGGHVVEGLAGELEQLRARLEHHPQGGSHHHHHH

SEQ ID NO: 58 - protein, 375 aa, synthetic construct
MRVPFTELQSLLQAIFQRHGCSEAVARVLAHNCASAQRDGAHSHGVFRMPGYVSTLASGWVDGQATPQVSDVAAGYVRVDAAGGFAQPALAAARELLVAKARSAGIAVLAIHNSHHFAALWPDVEPFAEEGLVALSVVNSYTCVVPHGARKPLFGTNPIAFAAPCAEHDPIVFDMATSAMAMGDVQIAARAGQQLPEGMGVDADGQPTTDPKAILEGGALLPFGGHKGSALSMMVELLAAALTGGHFSWEFDWSGHPGAETPWTGQLIIVIDPGKAEGQRFAQRSRELVEHMQAVGLTRMPGERRYREREVAEEEGVAVTEQELKGLKELLGGTDEKTTGWRGGHVVEGLAGELEQLRARLEHHPQGGSHHHHHH

SEQ ID NO: 59 - protein, 375 aa, synthetic construct
MRVPFTELQSLLQAIFQRHGCSEAVARVLAHNCASAQRDGAHSHGVFRMPGYVSTLASGWVDGQATPQVSDVAAGYVRVDAAGGFAQPALAAARELLVAKARSAGIAVLAIHNSHHFAALWPDVEPFAEEGLVALSVVNSYTCVVPHGARKPLFGTNPIAFAAPCAEHDPIVFDMATSAMAMGDVQIAARAGQQLPEGMGVDADGQPTTDPKAILEGGALLPFGGHKGSALSMMVELLAAALTGGHFSWEFDWSGHPGAQTPWTGQLIIVIDPGKAEGQRFAQRSRELVEHMQAVGLTRMPGERRYREREVAEEEGVAVTEQELKGLKELLGGTDEKTTGWRGGHVVEGLAGELEQLRARLEHHPQGGSHHHHHH

SEQ ID NO: 60 - protein, 375 aa, synthetic construct
MRVPFTELQSLLQAIFQRHGCSEAVARVLAHNCASAQRDGAHSHGVFRMPGYVSTLASGWVDGQATPQVSDVAAGYVRVDAAGGFAQPALAAARELLVAKARSAGIAVLAIHNSHHFAALWPDVEPFAEEGLVALSVVNSMTCVVPHGARKPLFGTNPIAFAAPCAEHDPIVFDMATSAMALGDVQIAARAGQQLPEGMGVDADGQPTTDPKAILEGGALLPFGGHKGSALSMMVELLAAALTGGHFSWEFDHSGHPGAETPWTGQLIIVIDPGKAEGQRFAQRSRELVEHMQAVGLTRMPGERRYREREVAEEEGVAVTEQELKGLKELLGGTDEKTTGWRGGHVVEGLAGELEQLRARLEHHPQGGSHHHHHH

SEQ ID NO: 61 - protein, 375 aa, synthetic construct
MRVPFTELQSLLQAIFQRHGCSEAVARVLAHNCASAQRDGAHSHGVFRMPGYVSTLASGWVDGQATPQVSDVAAGYVRVDAAGGFAQPALAAARELLVAKARSAGIAVLAIHNSHHFAALWPDVEPFAEEGLVALSVVNSMTCVVPHGARKPLFGTNPIAFAAPCAEHDPIVFDMATSAMALGDVQIAARAGQQLPEGMGVDADGQPTTDPKAILEGGALLPFGGHKGSALSMMVELLAAALTGGHFSWEFDMSGHPGAETPWTGQLIIVIDPGKAEGQRFAQRSRELVEHMQAVGLTRMPGERRYREREVAEEEGVAVTEQELKGLKELLGGTDEKTTGWRGGHVVEGLAGELEQLRARLEHHPQGGSHHHHHH

SEQ ID NO: 62 - protein, 375 aa, synthetic construct
MRVPFTELQSLLQAIFQRHGCSEAVARVLAHNCASAQRDGAHSHGVFRMPGYVSTLASGWVDGQATPQVSDVAAGYVRVDAAGGFAQPALAAARELLVAKARSAGIAVLAIHNSHHFAALWPDVEPFAEEGLVALSVVNSMTCVVPHGARKPLFGTNPIAFAAPCAEHDPIVFDMATSAMALGDVQIAARAGQQLPEGMGVDADGQPTTDPKAILEGGALLPFGGHKGSALSMMVELLAAALTGGHFSWEFDQSGHPGAETPWTGQLIIVIDPGKAEGQRFAQRSRELVEHMQAVGLTRMPGERRYREREVAEEEGVAVTEQELKGLKELLGGTDEKTTGWRGGHVVEGLAGELEQLRARLEHHPQGGSHHHHHH